European Patent Application EP 4 169 948 A1, published April 26, 2023. Title: Anti-CD73 antibody and uses thereof. Applicant: INNOVENT BIOLOGICS (SUZHOU) CO., LTD. The sequence listing filed with the application follows.

SEQUENCE LISTING (156 sequences)

SEQ ID NO: 1 - protein, 10 aa, artificial sequence
  Synthetic
GFTFDDYAMH

SEQ ID NO: 2 - protein, 10 aa, artificial sequence
  Synthetic
GFTFDDFYMH

SEQ ID NO: 3 - protein, 10 aa, artificial sequence
  Synthetic
GFTFDDYFMH

SEQ ID NO: 4 - protein, 10 aa, artificial sequence
  Synthetic
GFTFSNYAMS

SEQ ID NO: 5 - protein, 10 aa, artificial sequence
  Synthetic
GFTFHNYAMS

SEQ ID NO: 6 - protein, 10 aa, artificial sequence
  Synthetic
GFTFSNYAMT

SEQ ID NO: 7 - protein, 10 aa, artificial sequence
  Synthetic
GFTFSNLAMS

SEQ ID NO: 8 - protein, 10 aa, artificial sequence
  Synthetic
GFTFLNYAMA

SEQ ID NO: 9 - protein, 10 aa, artificial sequence
  Synthetic
GFTFSSYGMH

SEQ ID NO: 10 - protein, 10 aa, artificial sequence
  Synthetic
GFTFNFYGMH

SEQ ID NO: 11 - protein, 10 aa, artificial sequence
  Synthetic
GFTFSHYGMH

SEQ ID NO: 12 - protein, 10 aa, artificial sequence
  Synthetic
GFTFSSYSMH

SEQ ID NO: 13 - protein, 11 aa, artificial sequence
  Synthetic
GYSISSGYYWG

SEQ ID NO: 14 - protein, 11 aa, artificial sequence
  Synthetic
GYSISEGYYWG

SEQ ID NO: 15 - protein, 11 aa, artificial sequence
  Synthetic
GYSISSGYYWA

SEQ ID NO: 16 - protein, 17 aa, artificial sequence
  Synthetic
GISWSSGSIGYADSVKG

SEQ ID NO: 17 - protein, 17 aa, artificial sequence
  Synthetic
GISWSSTSIDYADSVKG

SEQ ID NO: 18 - protein, 17 aa, artificial sequence
  Synthetic
GISWSSGPIDYADSVKG

SEQ ID NO: 19 - protein, 17 aa, artificial sequence
  Synthetic
AISGSGGSTYYADSVKG

SEQ ID NO: 20 - protein, 17 aa, artificial sequence
  Synthetic
AISGRASSTYYADSVKG

SEQ ID NO: 21 - protein, 17 aa, artificial sequence
  Synthetic
AISGTGRATYYADSVKG

SEQ ID NO: 22 - protein, 17 aa, artificial sequence
  Synthetic
AISGRGTATYYADSVKG

SEQ ID NO: 23 - protein, 17 aa, artificial sequence
  Synthetic
AISGRATSTYYADSVKG

SEQ ID NO: 24 - protein, 17 aa, artificial sequence
  Synthetic
VISYEGSNKYYADSVKG

SEQ ID NO: 25 - protein, 17 aa, artificial sequence
  Synthetic
VINDEGINKYYADSVKG

SEQ ID NO: 26 - protein, 17 aa, artificial sequence
  Synthetic
VISDEGSNKYYADSVKG

SEQ ID NO: 27 - protein, 16 aa, artificial sequence
  Synthetic
HIVEGSDKYYADSVKG

SEQ ID NO: 28 - protein, 16 aa, artificial sequence
  Synthetic
SIYHSGSTYYNPSLKS

SEQ ID NO: 29 - protein, 16 aa, artificial sequence
  Synthetic
SIYHTGFTYYNPSLKS

SEQ ID NO: 30 - protein, 16 aa, artificial sequence
  Synthetic
SIFHSGFTFYNPSLKS

SEQ ID NO: 31 - protein, 14 aa, artificial sequence
  Synthetic
AKDRRYGLTYGMDV

SEQ ID NO: 32 - protein, 13 aa, artificial sequence
  Synthetic
AKGKYLPTGSVDY

SEQ ID NO: 33 - protein, 17 aa, artificial sequence
  Synthetic
ARGGPYGSGSYWDTFDY

SEQ ID NO: 34 - protein, 13 aa, artificial sequence
  Synthetic
ARGGARYPIAFDI

SEQ ID NO: 35 - protein, 13 aa, artificial sequence
  Synthetic
ARGWLRYPIAFDI

SEQ ID NO: 36 - protein, 12 aa, artificial sequence
  Synthetic
ARSRYDWSLFDI

SEQ ID NO: 37 - protein, 15 aa, artificial sequence
  Synthetic
ARASIYTPPPEYFQH

SEQ ID NO: 38 - protein, 11 aa, artificial sequence
  Synthetic
QASQDITNYLN

SEQ ID NO: 39 - protein, 12 aa, artificial sequence
  Synthetic
RASQSVSSSYLA

SEQ ID NO: 40 - protein, 11 aa, artificial sequence
  Synthetic
RASQSVSSNLA

SEQ ID NO: 41 - protein, 11 aa, artificial sequence
  Synthetic
RASQDISSWLA

SEQ ID NO: 42 - protein, 12 aa, artificial sequence
  Synthetic
GASQSVSSSYLA

SEQ ID NO: 43 - protein, 11 aa, artificial sequence
  Synthetic
RASQSISSWLA

SEQ ID NO: 44 - protein, 7 aa, artificial sequence
  Synthetic
DASNLET

SEQ ID NO: 45 - protein, 7 aa, artificial sequence
  Synthetic
GASSRAT

SEQ ID NO: 46 - protein, 7 aa, artificial sequence
  Synthetic
GASTRAT

SEQ ID NO: 47 - protein, 7 aa, artificial sequence
  Synthetic
AASSLQS

SEQ ID NO: 48 - protein, 7 aa, artificial sequence
  Synthetic
DASSLES

SEQ ID NO: 49 - protein, 9 aa, artificial sequence
  Synthetic
QQSVVLPFT

SEQ ID NO: 50 - protein, 10 aa, artificial sequence
  Synthetic
QQYYDYPPIT

SEQ ID NO: 51 - protein, 8 aa, artificial sequence
  Synthetic
QQYTNHYT

SEQ ID NO: 52 - protein, 9 aa, artificial sequence
  Synthetic
QQANDFPIT

SEQ ID NO: 53 - protein, 9 aa, artificial sequence
  Synthetic
QQYVLYPFT

SEQ ID NO: 54 - protein, 8 aa, artificial sequence
  Synthetic
QQSRIYST

SEQ ID NO: 55 - protein, 121 aa, artificial sequence
  Synthetic
EVQLVESGGGLVQPGRSLRLSCAASGFTFDDYAMHWVRQAPGKGLEWVSGISWSSGSIGYADSVKGRFTISRDNAKNSLYLQMNSLRAEDTAVYYCAKDRRYGLTYGMDVWGQGTTVTVSS

SEQ ID NO: 56 - protein, 120 aa, artificial sequence
  Synthetic
EVQLVESGGGLVQPGRSLRLSCAASGFTFDDYAMHWVRQAPGKGLEWVSGISWSSGSIGYADSVKGRFTISRDNAKNSLYLQMNSLRAEDTAVYYCAKGKYLPTGSVDYWGQGTLVTVSS

SEQ ID NO: 57 - protein, 120 aa, artificial sequence
  Synthetic
EVQLVESGGGLVQPGRSLRLSCAASGFTFDDFYMHWVRQAPGKGLEWVSGISWSSTSIDYADSVKGRFTISRDNAKNSLYLQMNSLRAEDTAVYYCAKGKYLPTGSVDYWGQGTLVTVSS

SEQ ID NO: 58 - protein, 120 aa, artificial sequence
  Synthetic
EVQLVESGGGLVQPGGSLRLSCAASGFTFDDYFMHWVRQAPGKGLEWVSGISWSSGPIDYADSVKGRFTISRDNAKNSLYLQMNSLRAEDTAVYYCAKGKYLPTGSVDYWGQGTLVTVSS

SEQ ID NO: 59 - protein, 124 aa, artificial sequence
  Synthetic
EVQLLESGGGLVQPGGSLRLSCAASGFTFSNYAMSWVRQAPGKGLEWVSAISGSGGSTYYADSVKGRFTISRDNSKNTLYLQMNSLRAEDTAVYYCARGGPYGSGSYWDTFDYWGQGTLVTVSS

SEQ ID NO: 60 - protein, 124 aa, artificial sequence
  Synthetic
EVQLLESGGGLVQPGGSLRLSCAASGFTFSNYAMSWVRQAPGKGLEWVSAISGRASSTYYADSVKGRFTISRDNSKNTLYLQMNSLRAEDTAVYYCARGGPYGSGSYWDTFDYWGQGTLVTVSS

SEQ ID NO: 61 - protein, 124 aa, artificial sequence
  Synthetic
EVQLLESGGGLVQPGGSLRLSCAASGFTFHNYAMSWVRQAPGKGLEWVSAISGTGRATYYADSVKGRFTISRDNSKNTLYLQMNSLRAEDTAVYYCARGGPYGSGSYWDTFDYWGQGTLVTVSS

SEQ ID NO: 62 - protein, 124 aa, artificial sequence
  Synthetic
QVQLVESGGGLVQPGGSLRLSCAASGFTFSNYAMTWVRQAPGKGLEWVSAISGRGTATYYADSVKGRFTISRDNSKNTLYLQMNSLRAEDTAVYYCARGGPYGSGSYWDTFDYWGQGTLVTVSS

SEQ ID NO: 63 - protein, 124 aa, artificial sequence
  Synthetic
EVQLLESGGGLVQPGGSLRLSCAASGFTFSNLAMSWVRQAPGKGLEWVSAISGRATSTYYADSVKGRFTISRDNSKNTLYLQMNSLRAEDTAVYYCARGGPYGSGSYWDTFDYWGQGTLVTVSS

SEQ ID NO: 64 - protein, 124 aa, artificial sequence
  Synthetic
EVQLLESGGGLVQPGGSLRLSCAASGFTFLNYAMAWVRQAPGKGLEWVSAISGRATSTYYADSVKGRFTISRDNSKNTLYLQMNSLRAEDTAVYYCARGGPYGSGSYWDTFDYWGQGTLVTVSS

SEQ ID NO: 65 - protein, 120 aa, artificial sequence
  Synthetic
QVQLVESGGGVVQPGRSLRLSCAASGFTFSSYGMHWVRQAPGKGLEWVAVISYEGSNKYYADSVKGRFTISRDNSKNTLYLQMNSLRAEDTAVYYCARGGARYPIAFDIWGQGTMVTVSS

SEQ ID NO: 66 - protein, 120 aa, artificial sequence
  Synthetic
EVQLLESGGGVVQPGRSLRLSCAASGFTFNFYGMHWVRQAPGKGLEWVAVINDEGINKYYADSVKGRFTISRDNSKNTLYLQMNSLRAEDTAVYYCARGGARYPIAFDIWGQGTMVTVSS

SEQ ID NO: 67 - protein, 120 aa, artificial sequence
  Synthetic
QVQLVESGGGVVQPGRSLRLSCAASGFTFSHYGMHWVRQAPGKGLEWVAVISDEGSNKYYADSVKGRFTISRDNSKNTLYLQMNSLRAEDTAVYYCARGWLRYPIAFDIWGQGTMVTVSS

SEQ ID NO: 68 - protein, 119 aa, artificial sequence
  Synthetic
QVQLVESGGGVVQPGRSLRLSCAASGFTFSSYGMHWVRQAPGKGLEWVAVISYEGSNKYYADSVKGRFTISRDNSKNTLYLQMNSLRAEDTAVYYCARSRYDWSLFDIWGQGTMVTVSS

SEQ ID NO: 69 - protein, 118 aa, artificial sequence
  Synthetic
QVQLVESGGGVVQPGRSLRLSCAASGFTFSSYSMHWVRQAPGKGLEWVAHIVEGSDKYYADSVKGRFTISRDNSKNTLYLQMNSLRAEDTAVYYCARSRYDWSLFDIWGQGTMVTVSS

SEQ ID NO: 70 - protein, 122 aa, artificial sequence
  Synthetic
QVQLQESGPGLVKPSETLSLTCAVSGYSISSGYYWGWIRQPPGKGLEWIGSIYHSGSTYYNPSLKSRVTISVDTSKNQFSLKLSSVTAADTAVYYCARASIYTPPPEYFQHWGQGTLVTVSS

SEQ ID NO: 71 - protein, 122 aa, artificial sequence
  Synthetic
QVQLQESGPGLVKPSETLSLTCAVSGYSISEGYYWGWIRQPPGKGLEWIGSIYHTGFTYYNPSLKSRVTISVDTSKNQFSLKLSSVTAADTAVYYCARASIYTPPPEYFQHWGQGTLVTVSS

SEQ ID NO: 72 - protein, 122 aa, artificial sequence
  Synthetic
QVQLQESGPGLVKPSETLSLTCAVSGYSISSGYYWAWIRQPPGKGLEWIGSIFHSGFTFYNPSLKSRVTISVDTSKNQFSLKLSSVTAADTAVYYCARASIYTPPPEYFQHWGQGTLVTVSS

SEQ ID NO: 73 - DNA, 363 bp, artificial sequence
  Synthetic
gaagtgcagctggtggagtctgggggaggcttggtacagcctggcaggtccctgagactctcctgtgcagcctctggattcacctttgatgattatgccatgcactgggtccggcaagctccagggaagggcctggagtgggtctcaggtattagttggagtagtggtagcataggctatgcggactctgtgaagggccgattcaccatctccagagacaacgccaagaactccctgtatctgcaaatgaacagtctgagagctgaggacacggcggtgtactactgcgccaaggacagaagatacggcttaacatacggaatggacgtatggggccagggaacaactgtcaccgtctcctca

SEQ ID NO: 74 - DNA, 360 bp, artificial sequence
  Synthetic
gaagtgcagctggtggagtctgggggaggcttggtacagcctggcaggtccctgagactctcctgtgcagcctctggattcacctttgatgattatgccatgcactgggtccggcaagctccagggaagggcctggagtgggtctcaggtattagttggagtagtggtagcataggctatgcggactctgtgaagggccgattcaccatctccagagacaacgccaagaactccctgtatctgcaaatgaacagtctgagagctgaggacacggcggtgtactactgcgcaaagggcaagtatctaccaaccggaagcgtggactactggggacagggtacattggtaaccgtctcctca

SEQ ID NO: 75 - DNA, 360 bp, artificial sequence
  Synthetic
gaagtgcagctggtggagtctgggggaggcttggtacagcctggcaggtccctgagactctcctgtgcagcctctggattcacctttgatgatttctacatgcactgggtccggcaagctccagggaagggcctggagtgggtctcaggtattagttggagtagtaccagcatagactatgcggactctgtgaagggccggttcaccatctccagagacaacgccaagaactccctgtatctgcaaatgaacagcctgagagccgaggacacggcggtgtactactgcgcaaagggcaagtatctaccaaccggaagcgtggactactggggacagggtacattggtaaccgtctcctca

SEQ ID NO: 76 - DNA, 360 bp, artificial sequence
  Synthetic
gaggtgcagctggtggagtctgggggaggcttggtccagcctggggggtccctgagactctcctgtgcagcctctggattcacctttgatgattatttcatgcactgggtccggcaagctccagggaagggcctggagtgggtctcaggtattagttggagtagtggtcccatagactatgcggactctgtgaagggccgattcaccatctccagagacaacgccaagaactccctgtatctgcaaatgaacagtctgagagctgaggacacggcggtgtactactgcgcaaagggcaagtatctaccaaccggaagcgtggactactggggacagggtacattggtaaccgtctcctca

SEQ ID NO: 77 - DNA, 372 bp, artificial sequence
  Synthetic
gaggtgcagctgttggagtctgggggaggcttggtacagcctggggggtccctgagactctcctgtgcagcctctggattcacctttagcaattatgccatgagctgggtccgccaggctccagggaaggggctggagtgggtctcagctattagtggtagtggtggtagcacatactacgcagactccgtgaagggccggttcaccatctccagagacaattccaagaacacgctgtatctgcaaatgaacagcctgagagccgaggacacggcggtgtactactgcgccagaggtgggccttacggaagcggaagctactgggatacctttgattattggggacagggtacattggtcaccgtctcctca

SEQ ID NO: 78 - DNA, 372 bp, artificial sequence
  Synthetic
gaggtgcagctgttggagtctgggggaggcttggtacagcctggggggtccctgagactctcctgtgcagcctctggattcacctttagcaattatgccatgagctgggtccgccaggctccagggaaagggctggagtgggtctcagctattagtggacgagcatccagcacatactacgcagactccgtgaagggccggttcaccatctccagagacaattccaagaacacgctgtatctgcaaatgaacagcctgagagccgaggacacggcggtgtactactgcgccagaggtgggccttacggaagcggaagctactgggatacctttgattattggggacagggtacattggtcaccgtctcctca

SEQ ID NO: 79 - DNA, 372 bp, artificial sequence
  Synthetic
gaggtgcagctgttggagtctgggggaggcttggtacagcctggggggtccctgagactctcctgtgcagcctctggattcacctttcacaactatgccatgagctgggtccgccaggctccagggaaggggctggagtgggtctcagctattagtggtacaggtagagcaacatactacgcagactccgtgaagggccggttcaccatctccagagacaattccaagaacacgctgtatctgcaaatgaacagcctgagagccgaggacacggcggtgtactactgcgccagaggtgggccttacggaagcggaagctactgggatacctttgattattggggacagggtacattggtcaccgtctcctca

SEQ ID NO: 80 - DNA, 372 bp, artificial sequence
  Synthetic
caggtgcagctggtggagtctgggggaggcttggtacagcctggggggtccctgagactctcctgtgcagcctctggattcacctttagcaactatgccatgacctgggtccgccaggctccagggaaggggctggagtgggtctcagctattagtggtagaggtacagcaacatactacgcagactccgtgaagggccgattcaccatctccagagacaattccaagaacacgctgtatctgcaaatgaacagcctgagagccgaggacacggcggtgtactactgcgccagaggtgggccttacggaagcggaagctactgggatacctttgattattggggacagggtacattggtcaccgtctcctca

SEQ ID NO: 81 - DNA, 372 bp, artificial sequence
  Synthetic
gaggtgcagctgttggagtctgggggaggcttggtacagcctggggggtccctgagactctcctgtgcagcctctggattcacctttagcaacctcgccatgtcctgggtccgccaggctccagggaaggggctggagtgggtctcagctattagtggacgagcaacaagcacatactacgcagactccgtgaagggccggttcaccatctccagagacaattccaagaacacgctgtatctgcaaatgaacagcctgagagccgaggacacggcggtgtactactgcgccagaggtgggccttacggaagcggaagctactgggatacctttgattattggggacagggtacattggtcaccgtctcctca

SEQ ID NO: 82 - DNA, 372 bp, artificial sequence
  Synthetic
gaggtgcagctgttggagtctgggggaggcttggtacagcctggggggtccctgagactctcctgtgcagcctctggattcacctttctcaactatgccatggcctgggtccgccaggctccagggaaggggctggagtgggtctcagctattagtggaagagcaacaagcacatactacgcagactccgtgaagggccggttcaccatctccagagacaattccaagaacacgctgtatctgcaaatgaacagcctgagagccgaggacacggcggtgtactactgcgccagaggtgggccttacggaagcggaagctactgggatacctttgattattggggacagggtacattggtcaccgtctcctca

SEQ ID NO: 83 - DNA, 360 bp, artificial sequence
  Synthetic
caggtgcagctggtggagtctgggggaggcgtggtccagcctgggaggtccctgagactctcctgtgcagcgtctggattcaccttcagtagctatggcatgcactgggtccgccaggctccaggcaaggggctggagtgggtggcagttatatcgtatgagggaagtaataaatactatgcagactccgtgaagggccgattcaccatctccagagacaattccaagaacacgctgtatctgcaaatgaacagcctgagagccgaggacacggcggtgtactactgcgccagaggaggtgctagatacccaatagcattcgacatatggggtcagggtacaatggtcaccgtctcctca

SEQ ID NO: 84 - DNA, 360 bp, artificial sequence
  Synthetic
gaggtgcagctgttggagtctgggggaggcgtggtccagcctgggaggtccctgagactctcctgtgcagcgtctggattcaccttcaacttctatggcatgcactgggtccgccaggctccaggcaaggggctggagtgggtggcagttataaacgacgagggaatcaataaatactatgcagactccgtgaagggccgattcaccatctccagagacaattccaagaacacgctgtatctgcaaatgaacagcctgagagccgaggacacggcggtgtactactgcgccagaggaggtgctagatacccaatagcattcgacatatggggtcagggtacaatggtcaccgtctcctca

SEQ ID NO: 85 - DNA, 360 bp, artificial sequence
  Synthetic
caggtgcagctggtggagtctgggggaggcgtggtccagcctgggaggtccctgagactctcctgtgcagcgtctggattcaccttcagtcactatggcatgcactgggtccgccaggctccaggcaaggggctggagtgggtggcagttatatcggacgagggatccaataaatactatgcagactccgtgaagggccgattcaccatctccagagacaattccaagaacacgctgtatctgcaaatgaacagcctgagagccgaggacacggcggtgtactactgcgccagaggatggcttagatacccaatagcattcgacatatggggtcagggtacaatggtcaccgtctcctca

SEQ ID NO: 86 - DNA, 357 bp, artificial sequence
  Synthetic
caggtgcagctggtggagtctgggggaggcgtggtccagcctgggaggtccctgagactctcctgtgcagcgtctggattcaccttcagtagctatggcatgcactgggtccgccaggctccaggcaaggggctggagtgggtggcagttatatcgtatgagggaagtaataaatactatgcagactccgtgaagggccgattcaccatctccagagacaattccaagaacacgctgtatctgcaaatgaacagcctgagagccgaggacacggcggtgtactactgcgctagatcaagatacgactggagtctattcgacatatggggtcagggtacaatggtcaccgtctcctca

SEQ ID NO: 87 - DNA, 354 bp, artificial sequence
  Synthetic
caggtgcagctggtggagtctgggggaggcgtggtccagcctgggaggtccctgagactctcctgtgcagcgtctggattcaccttctccagctattccatgcactgggtccgccaggctccaggcaaggggctggagtgggtggcacatatcgtagagggaagtgacaaatactatgcagactccgtgaagggccgattcaccatctccagagacaattccaagaacacgctgtatctgcaaatgaacagcctgagagccgaggacacggcggtgtactactgcgctagatcaagatacgactggagtctattcgacatatggggtcagggtacaatggtcaccgtctcctca

SEQ ID NO: 88 - DNA, 366 bp, artificial sequence
  Synthetic
caggtgcagctgcaggagtcgggcccaggactggtgaagccttcggagaccctgtccctcacctgcgctgtctctggttactccatcagcagtggttactactggggctggatccggcagcccccagggaaggggctggagtggattgggagtatctatcatagtgggagcacctactacaacccgtccctcaagagtcgagtcaccatatcagtagacacgtccaagaaccagttctccctgaagctgagttctgtgaccgccgcagacacggcggtgtactactgcgctagggcatctatatacactccacctccagaatacttccaacactggggacagggtacattggtcaccgtctcctca

SEQ ID NO: 89 - DNA, 366 bp, artificial sequence
  Synthetic
caggtgcagctgcaggagtcgggcccaggactggtgaagccttcggagaccctgtccctcacctgcgctgtctctggttactccatcagcgaaggttactactggggctggatccggcagcccccagggaaggggctggagtggattgggagtatctatcatacagggttcacctactacaacccgtccctcaagagtcgagtcaccatatcagtagacacgtccaagaaccagttctccctgaagctgagctctgtgaccgccgcagacacggcggtgtactactgcgctagggcatctatatacactccacctccagaatacttccaacactggggacagggtacattggtcaccgtctcctca

SEQ ID NO: 90 - DNA, 366 bp, artificial sequence
  Synthetic
caggtgcagctgcaggagtcgggcccaggactggtgaagccttcggagaccctgtccctcacctgcgctgtctctggttactccatctccagtggttactactgggcctggatccggcagcccccagggaaggggctggagtggattgggagtatcttccatagtgggttcaccttctacaacccgtccctcaagagtcgagtcaccatatcagtagacacgtccaagaaccagttctccctgaagctgagttctgtgaccgccgcagacacggcggtgtactactgcgctagggcatctatatacactccacctccagaatacttccaacactggggacagggtacattggtcaccgtctcctca

SEQ ID NO: 91 - protein, 107 aa, artificial sequence
  Synthetic
DIQMTQSPSSLSASVGDRVTITCQASQDITNYLNWYQQKPGKAPKLLIYDASNLETGVPSRFSGSGSGTDFTFTISSLQPEDIATYYCQQSVVLPFTFGGGTKVEIK

SEQ ID NO: 92 - protein, 109 aa, artificial sequence
  Synthetic
EIVLTQSPGTLSLSPGERATLSCRASQSVSSSYLAWYQQKPGQAPRLLIYGASSRATGIPDRFSGSGSGTDFTLTISRLEPEDFAVYYCQQYYDYPPITFGGGTKVEIK

SEQ ID NO: 93 - protein, 106 aa, artificial sequence
  Synthetic
EIVMTQSPATLSVSPGERATLSCRASQSVSSNLAWYQQKPGQAPRLLIYGASTRATGIPARFSGSGSGTEFTLTISSLQSEDFAVYYCQQYTNHYTFGGGTKVEIK

SEQ ID NO: 94 - protein, 107 aa, artificial sequence
  Synthetic
DIQLTQSPSSVSASVGDRVTITCRASQDISSWLAWYQQKPGKAPKLLIYAASSLQSGVPSRFSGSGSGTDFTLTISSLQPEDFATYYCQQANDFPITFGGGTKVEIK

SEQ ID NO: 95 - protein, 108 aa, artificial sequence
  Synthetic
EIVLTQSPGTLSLSPGERATLSCRASQSVSSSYLAWYQQKPGQAPRLLIYGASSRATGIPDRFSGSGSGTDFTLTISRLEPEDFAVYYCQQYVLYPFTFGGGTKVEIK

SEQ ID NO: 96 - protein, 108 aa, artificial sequence
  Synthetic
EIVLTQSPGTLSLSPGERATLSCGASQSVSSSYLAWYQQKPGQAPRLLIYGASSRATGIPDRFSGSGSGTDFTLTISRLEPEDFAVYYCQQYVLYPFTFGGGTKVEIK

SEQ ID NO: 97 - protein, 106 aa, artificial sequence
  Synthetic
DIQMTQSPSTLSASVGDRVTITCRASQSISSWLAWYQQKPGKAPKLLIYDASSLESGVPSRFSGSGSGTEFTLTISSLQPDDFATYYCQQSRIYSTFGGGTKVEIK

SEQ ID NO: 98 - DNA, 321 bp, artificial sequence
  Synthetic
gacatccagatgacccagtctccatcctccctgtctgcatctgtaggagacagagtcaccatcacttgccaggcgagtcaggacattaccaactatttaaattggtatcagcagaaaccagggaaagcccctaagctcctgatctacgatgcatccaatttggaaacaggggtcccatcaaggttcagtggaagtggatctgggacagattttactttcaccatcagcagcctgcagcctgaagatattgcaacatattactgtcagcagtccgtcgtcctccctttcacttttggcggagggaccaaggttgagatcaaa

SEQ ID NO: 99 - DNA, 327 bp, artificial sequence
  Synthetic
gaaattgtgttgacgcagtctccaggcaccctgtctttgtctccaggggaaagagccaccctctcctgcagggccagtcagagtgttagcagcagctacttagcctggtaccagcagaaacctggccaggctcccaggctcctcatctatggtgcatccagcagggccactggcatcccagacaggttcagtggcagtgggtctgggacagacttcactctcaccatcagcagactggagcctgaagattttgcagtgtattactgtcagcagtactacgactaccctcctatcacttttggcggagggaccaaggttgagatcaaa

SEQ ID NO: 100 - DNA, 318 bp, artificial sequence
  Synthetic
gaaatagtgatgacgcagtctccagccaccctgtctgtgtctccaggggaaagagccaccctctcctgcagggccagtcagagtgttagcagcaacttagcctggtaccagcagaaacctggccaggctcccaggctcctcatctatggtgcatccaccagggccactggtatcccagccaggttcagtggcagtgggtctgggacagagttcactctcaccatcagcagcctgcagtctgaagattttgcagtttattactgtcagcagtacaccaatcactacacttttggcggagggaccaaggttgagatcaaa

SEQ ID NO: 101 - DNA, 321 bp, artificial sequence
  Synthetic
gacatccagttgacccagtctccatcttccgtgtctgcatctgtaggagacagagtcaccatcacttgtcgggcgagtcaggatattagcagctggttagcctggtatcagcagaaaccagggaaagcccctaagctcctgatctatgctgcatccagtttgcaaagtggggtcccatcaaggttcagcggcagtggatctgggacagatttcactctcaccatcagcagcctgcagcctgaagattttgcaacttactactgtcagcaggcaaatgacttccctatcacttttggcggagggaccaaggttgagatcaaa

SEQ ID NO: 102 - DNA, 324 bp, artificial sequence
  Synthetic
gaaattgtgttgacgcagtctccaggcaccctgtctttgtctccaggggaaagagccaccctctcctgcagggccagtcagagtgttagcagcagctacttagcctggtaccagcagaaacctggccaggctcccaggctcctcatctatggtgcatccagcagggccactggcatcccagacaggttcagtggcagtgggtctgggacagacttcactctcaccatcagcagactggagcctgaagattttgcagtgtattactgtcagcagtacgtcctctaccctttcacttttggcggagggaccaaggttgagatcaaa

SEQ ID NO: 103 - DNA, 324 bp, artificial sequence
  Synthetic
gaaattgtgttgacgcagtctccaggcaccctgtctttgtctccaggggaaagagccaccctctcctgcggggccagtcagagtgttagcagcagctacttagcctggtaccagcagaaacctggccaggctcccaggctcctcatctatggtgcatccagcagggccactggcatcccagacaggttcagtggcagtgggtctgggacagacttcactctcaccatcagcagactggagcctgaagattttgcagtgtattactgtcagcagtacgtcctctaccctttcacttttggcggagggaccaaggttgagatcaaa

SEQ ID NO: 104 - DNA, 318 bp, artificial sequence
  Synthetic
gacatccagatgacccagtctccttccaccctgtctgcatctgtaggagacagagtcaccatcacttgccgggccagtcagagtattagtagctggttggcctggtatcagcagaaaccagggaaagcccctaagctcctgatctatgatgcctccagtttggaaagtggggtcccatcaaggttcagcggcagtggatctgggacagaattcactctcaccatcagcagcctgcagcctgatgattttgcaacttattactgccagcagtccagaatctactctacttttggcggagggaccaaggttgagatcaaa

SEQ ID NO: 105 - DNA, 318 bp, artificial sequence
  Synthetic
gacatccagatgacccagtctccttccaccctgtctgcatctgtaggagacagagtcaccatcacttgccgggccagtcagagtattagtagctggttggcctggtatcagcagaaaccagggaaagcccctaagctcctgatctatgatgcctccagtttggaaagtggggtcccatcaaggttcagcggcagtggatctgggacagaattcactctcaccatcagcagcctgcagcctgatgattttgcaacttattactgccagcagtccagaatctactctactttcggcggagggaccaaggtggagatcaaa

SEQ ID NO: 106 - protein, 447 aa, artificial sequence
  Synthetic
EVQLVESGGGLVQPGRSLRLSCAASGFTFDDYAMHWVRQAPGKGLEWVSGISWSSGSIGYADSVKGRFTISRDNAKNSLYLQMNSLRAEDTAVYYCAKDRRYGLTYGMDVWGQGTTVTVSSASTKGPSVFPLAPCSRSTSESTAALGCLVKDYFPEPVTVSWNSGALTSGVHTFPAVLQSSGLYSLSSVVTVPSSSLGTKTYTCNVDHKPSNTKVDKRVESKYGPPCPPCPAPEAAGGPSVFLFPPKPKDTLMISRTPEVTCVVVDVSQEDPEVQFNWYVDGVEVHNAKTKPREEQFNSTYRVVSVLTVLHQDWLNGKEYKCKVSNKGLPSSIEKTISKAKGQPREPQVYTLPPSQEEMTKNQVSLTCLVKGFYPSDIAVEWESNGQPENNYKTTPPVLDSDGSFFLYSRLTVDKSRWQEGNVFSCSVMHEALHNHYTQKSLSLSLG

SEQ ID NO: 107 - protein, 446 aa, artificial sequence
  Synthetic
EVQLVESGGGLVQPGRSLRLSCAASGFTFDDYAMHWVRQAPGKGLEWVSGISWSSGSIGYADSVKGRFTISRDNAKNSLYLQMNSLRAEDTAVYYCAKGKYLPTGSVDYWGQGTLVTVSSASTKGPSVFPLAPCSRSTSESTAALGCLVKDYFPEPVTVSWNSGALTSGVHTFPAVLQSSGLYSLSSVVTVPSSSLGTKTYTCNVDHKPSNTKVDKRVESKYGPPCPPCPAPEAAGGPSVFLFPPKPKDTLMISRTPEVTCVVVDVSQEDPEVQFNWYVDGVEVHNAKTKPREEQFNSTYRVVSVLTVLHQDWLNGKEYKCKVSNKGLPSSIEKTISKAKGQPREPQVYTLPPSQEEMTKNQVSLTCLVKGFYPSDIAVEWESNGQPENNYKTTPPVLDSDGSFFLYSRLTVDKSRWQEGNVFSCSVMHEALHNHYTQKSLSLSLG

SEQ ID NO: 108 - protein, 446 aa, artificial sequence
  Synthetic
EVQLVESGGGLVQPGRSLRLSCAASGFTFDDFYMHWVRQAPGKGLEWVSGISWSSTSIDYADSVKGRFTISRDNAKNSLYLQMNSLRAEDTAVYYCAKGKYLPTGSVDYWGQGTLVTVSSASTKGPSVFPLAPCSRSTSESTAALGCLVKDYFPEPVTVSWNSGALTSGVHTFPAVLQSSGLYSLSSVVTVPSSSLGTKTYTCNVDHKPSNTKVDKRVESKYGPPCPPCPAPEAAGGPSVFLFPPKPKDTLMISRTPEVTCVVVDVSQEDPEVQFNWYVDGVEVHNAKTKPREEQFNSTYRVVSVLTVLHQDWLNGKEYKCKVSNKGLPSSIEKTISKAKGQPREPQVYTLPPSQEEMTKNQVSLTCLVKGFYPSDIAVEWESNGQPENNYKTTPPVLDSDGSFFLYSRLTVDKSRWQEGNVFSCSVMHEALHNHYTQKSLSLSLG

SEQ ID NO: 109 - protein, 446 aa, artificial sequence
  Synthetic
EVQLVESGGGLVQPGGSLRLSCAASGFTFDDYFMHWVRQAPGKGLEWVSGISWSSGPIDYADSVKGRFTISRDNAKNSLYLQMNSLRAEDTAVYYCAKGKYLPTGSVDYWGQGTLVTVSSASTKGPSVFPLAPCSRSTSESTAALGCLVKDYFPEPVTVSWNSGALTSGVHTFPAVLQSSGLYSLSSVVTVPSSSLGTKTYTCNVDHKPSNTKVDKRVESKYGPPCPPCPAPEAAGGPSVFLFPPKPKDTLMISRTPEVTCVVVDVSQEDPEVQFNWYVDGVEVHNAKTKPREEQFNSTYRVVSVLTVLHQDWLNGKEYKCKVSNKGLPSSIEKTISKAKGQPREPQVYTLPPSQEEMTKNQVSLTCLVKGFYPSDIAVEWESNGQPENNYKTTPPVLDSDGSFFLYSRLTVDKSRWQEGNVFSCSVMHEALHNHYTQKSLSLSLG

SEQ ID NO: 110 - protein, 450 aa, artificial sequence
  Synthetic
EVQLLESGGGLVQPGGSLRLSCAASGFTFSNYAMSWVRQAPGKGLEWVSAISGSGGSTYYADSVKGRFTISRDNSKNTLYLQMNSLRAEDTAVYYCARGGPYGSGSYWDTFDYWGQGTLVTVSSASTKGPSVFPLAPCSRSTSESTAALGCLVKDYFPEPVTVSWNSGALTSGVHTFPAVLQSSGLYSLSSVVTVPSSSLGTKTYTCNVDHKPSNTKVDKRVESKYGPPCPPCPAPEAAGGPSVFLFPPKPKDTLMISRTPEVTCVVVDVSQEDPEVQFNWYVDGVEVHNAKTKPREEQFNSTYRVVSVLTVLHQDWLNGKEYKCKVSNKGLPSSIEKTISKAKGQPREPQVYTLPPSQEEMTKNQVSLTCLVKGFYPSDIAVEWESNGQPENNYKTTPPVLDSDGSFFLYSRLTVDKSRWQEGNVFSCSVMHEALHNHYTQKSLSLSLG

SEQ ID NO: 111 - protein, 450 aa, artificial sequence
  Synthetic
EVQLLESGGGLVQPGGSLRLSCAASGFTFSNYAMSWVRQAPGKGLEWVSAISGRASSTYYADSVKGRFTISRDNSKNTLYLQMNSLRAEDTAVYYCARGGPYGSGSYWDTFDYWGQGTLVTVSSASTKGPSVFPLAPCSRSTSESTAALGCLVKDYFPEPVTVSWNSGALTSGVHTFPAVLQSSGLYSLSSVVTVPSSSLGTKTYTCNVDHKPSNTKVDKRVESKYGPPCPPCPAPEAAGGPSVFLFPPKPKDTLMISRTPEVTCVVVDVSQEDPEVQFNWYVDGVEVHNAKTKPREEQFNSTYRVVSVLTVLHQDWLNGKEYKCKVSNKGLPSSIEKTISKAKGQPREPQVYTLPPSQEEMTKNQVSLTCLVKGFYPSDIAVEWESNGQPENNYKTTPPVLDSDGSFFLYSRLTVDKSRWQEGNVFSCSVMHEALHNHYTQKSLSLSLG

SEQ ID NO: 112 - protein, 450 aa, artificial sequence
  Synthetic
EVQLLESGGGLVQPGGSLRLSCAASGFTFHNYAMSWVRQAPGKGLEWVSAISGTGRATYYADSVKGRFTISRDNSKNTLYLQMNSLRAEDTAVYYCARGGPYGSGSYWDTFDYWGQGTLVTVSSASTKGPSVFPLAPCSRSTSESTAALGCLVKDYFPEPVTVSWNSGALTSGVHTFPAVLQSSGLYSLSSVVTVPSSSLGTKTYTCNVDHKPSNTKVDKRVESKYGPPCPPCPAPEAAGGPSVFLFPPKPKDTLMISRTPEVTCVVVDVSQEDPEVQFNWYVDGVEVHNAKTKPREEQFNSTYRVVSVLTVLHQDWLNGKEYKCKVSNKGLPSSIEKTISKAKGQPREPQVYTLPPSQEEMTKNQVSLTCLVKGFYPSDIAVEWESNGQPENNYKTTPPVLDSDGSFFLYSRLTVDKSRWQEGNVFSCSVMHEALHNHYTQKSLSLSLG

SEQ ID NO: 113 - protein, 450 aa, artificial sequence
  Synthetic
QVQLVESGGGLVQPGGSLRLSCAASGFTFSNYAMTWVRQAPGKGLEWVSAISGRGTATYYADSVKGRFTISRDNSKNTLYLQMNSLRAEDTAVYYCARGGPYGSGSYWDTFDYWGQGTLVTVSSASTKGPSVFPLAPCSRSTSESTAALGCLVKDYFPEPVTVSWNSGALTSGVHTFPAVLQSSGLYSLSSVVTVPSSSLGTKTYTCNVDHKPSNTKVDKRVESKYGPPCPPCPAPEAAGGPSVFLFPPKPKDTLMISRTPEVTCVVVDVSQEDPEVQFNWYVDGVEVHNAKTKPREEQFNSTYRVVSVLTVLHQDWLNGKEYKCKVSNKGLPSSIEKTISKAKGQPREPQVYTLPPSQEEMTKNQVSLTCLVKGFYPSDIAVEWESNGQPENNYKTTPPVLDSDGSFFLYSRLTVDKSRWQEGNVFSCSVMHEALHNHYTQKSLSLSLG

SEQ ID NO: 114 - protein, 450 aa, artificial sequence
  Synthetic
EVQLLESGGGLVQPGGSLRLSCAASGFTFSNLAMSWVRQAPGKGLEWVSAISGRATSTYYADSVKGRFTISRDNSKNTLYLQMNSLRAEDTAVYYCARGGPYGSGSYWDTFDYWGQGTLVTVSSASTKGPSVFPLAPCSRSTSESTAALGCLVKDYFPEPVTVSWNSGALTSGVHTFPAVLQSSGLYSLSSVVTVPSSSLGTKTYTCNVDHKPSNTKVDKRVESKYGPPCPPCPAPEAAGGPSVFLFPPKPKDTLMISRTPEVTCVVVDVSQEDPEVQFNWYVDGVEVHNAKTKPREEQFNSTYRVVSVLTVLHQDWLNGKEYKCKVSNKGLPSSIEKTISKAKGQPREPQVYTLPPSQEEMTKNQVSLTCLVKGFYPSDIAVEWESNGQPENNYKTTPPVLDSDGSFFLYSRLTVDKSRWQEGNVFSCSVMHEALHNHYTQKSLSLSLG

SEQ ID NO: 115 - protein, 450 aa, artificial sequence
  Synthetic
EVQLLESGGGLVQPGGSLRLSCAASGFTFLNYAMAWVRQAPGKGLEWVSAISGRATSTYYADSVKGRFTISRDNSKNTLYLQMNSLRAEDTAVYYCARGGPYGSGSYWDTFDYWGQGTLVTVSSASTKGPSVFPLAPCSRSTSESTAALGCLVKDYFPEPVTVSWNSGALTSGVHTFPAVLQSSGLYSLSSVVTVPSSSLGTKTYTCNVDHKPSNTKVDKRVESKYGPPCPPCPAPEAAGGPSVFLFPPKPKDTLMISRTPEVTCVVVDVSQEDPEVQFNWYVDGVEVHNAKTKPREEQFNSTYRVVSVLTVLHQDWLNGKEYKCKVSNKGLPSSIEKTISKAKGQPREPQVYTLPPSQEEMTKNQVSLTCLVKGFYPSDIAVEWESNGQPENNYKTTPPVLDSDGSFFLYSRLTVDKSRWQEGNVFSCSVMHEALHNHYTQKSLSLSLG

SEQ ID NO: 116 - protein, 446 aa, artificial sequence
  Synthetic
QVQLVESGGGVVQPGRSLRLSCAASGFTFSSYGMHWVRQAPGKGLEWVAVISYEGSNKYYADSVKGRFTISRDNSKNTLYLQMNSLRAEDTAVYYCARGGARYPIAFDIWGQGTMVTVSSASTKGPSVFPLAPCSRSTSESTAALGCLVKDYFPEPVTVSWNSGALTSGVHTFPAVLQSSGLYSLSSVVTVPSSSLGTKTYTCNVDHKPSNTKVDKRVESKYGPPCPPCPAPEAAGGPSVFLFPPKPKDTLMISRTPEVTCVVVDVSQEDPEVQFNWYVDGVEVHNAKTKPREEQFNSTYRVVSVLTVLHQDWLNGKEYKCKVSNKGLPSSIEKTISKAKGQPREPQVYTLPPSQEEMTKNQVSLTCLVKGFYPSDIAVEWESNGQPENNYKTTPPVLDSDGSFFLYSRLTVDKSRWQEGNVFSCSVMHEALHNHYTQKSLSLSLG

SEQ ID NO: 117 - protein, 446 aa, artificial sequence
  Synthetic
EVQLLESGGGVVQPGRSLRLSCAASGFTFNFYGMHWVRQAPGKGLEWVAVINDEGINKYYADSVKGRFTISRDNSKNTLYLQMNSLRAEDTAVYYCARGGARYPIAFDIWGQGTMVTVSSASTKGPSVFPLAPCSRSTSESTAALGCLVKDYFPEPVTVSWNSGALTSGVHTFPAVLQSSGLYSLSSVVTVPSSSLGTKTYTCNVDHKPSNTKVDKRVESKYGPPCPPCPAPEAAGGPSVFLFPPKPKDTLMISRTPEVTCVVVDVSQEDPEVQFNWYVDGVEVHNAKTKPREEQFNSTYRVVSVLTVLHQDWLNGKEYKCKVSNKGLPSSIEKTISKAKGQPREPQVYTLPPSQEEMTKNQVSLTCLVKGFYPSDIAVEWESNGQPENNYKTTPPVLDSDGSFFLYSRLTVDKSRWQEGNVFSCSVMHEALHNHYTQKSLSLSLG

SEQ ID NO: 118 - protein, 446 aa, artificial sequence
  Synthetic
QVQLVESGGGVVQPGRSLRLSCAASGFTFSHYGMHWVRQAPGKGLEWVAVISDEGSNKYYADSVKGRFTISRDNSKNTLYLQMNSLRAEDTAVYYCARGWLRYPIAFDIWGQGTMVTVSSASTKGPSVFPLAPCSRSTSESTAALGCLVKDYFPEPVTVSWNSGALTSGVHTFPAVLQSSGLYSLSSVVTVPSSSLGTKTYTCNVDHKPSNTKVDKRVESKYGPPCPPCPAPEAAGGPSVFLFPPKPKDTLMISRTPEVTCVVVDVSQEDPEVQFNWYVDGVEVHNAKTKPREEQFNSTYRVVSVLTVLHQDWLNGKEYKCKVSNKGLPSSIEKTISKAKGQPREPQVYTLPPSQEEMTKNQVSLTCLVKGFYPSDIAVEWESNGQPENNYKTTPPVLDSDGSFFLYSRLTVDKSRWQEGNVFSCSVMHEALHNHYTQKSLSLSLG

SEQ ID NO: 119 - protein, 445 aa, artificial sequence
  Synthetic
QVQLVESGGGVVQPGRSLRLSCAASGFTFSSYGMHWVRQAPGKGLEWVAVISYEGSNKYYADSVKGRFTISRDNSKNTLYLQMNSLRAEDTAVYYCARSRYDWSLFDIWGQGTMVTVSSASTKGPSVFPLAPCSRSTSESTAALGCLVKDYFPEPVTVSWNSGALTSGVHTFPAVLQSSGLYSLSSVVTVPSSSLGTKTYTCNVDHKPSNTKVDKRVESKYGPPCPPCPAPEAAGGPSVFLFPPKPKDTLMISRTPEVTCVVVDVSQEDPEVQFNWYVDGVEVHNAKTKPREEQFNSTYRVVSVLTVLHQDWLNGKEYKCKVSNKGLPSSIEKTISKAKGQPREPQVYTLPPSQEEMTKNQVSLTCLVKGFYPSDIAVEWESNGQPENNYKTTPPVLDSDGSFFLYSRLTVDKSRWQEGNVFSCSVMHEALHNHYTQKSLSLSLG

SEQ ID NO: 120 - protein, 444 aa, artificial sequence
  Synthetic
QVQLVESGGGVVQPGRSLRLSCAASGFTFSSYSMHWVRQAPGKGLEWVAHIVEGSDKYYADSVKGRFTISRDNSKNTLYLQMNSLRAEDTAVYYCARSRYDWSLFDIWGQGTMVTVSSASTKGPSVFPLAPCSRSTSESTAALGCLVKDYFPEPVTVSWNSGALTSGVHTFPAVLQSSGLYSLSSVVTVPSSSLGTKTYTCNVDHKPSNTKVDKRVESKYGPPCPPCPAPEAAGGPSVFLFPPKPKDTLMISRTPEVTCVVVDVSQEDPEVQFNWYVDGVEVHNAKTKPREEQFNSTYRVVSVLTVLHQDWLNGKEYKCKVSNKGLPSSIEKTISKAKGQPREPQVYTLPPSQEEMTKNQVSLTCLVKGFYPSDIAVEWESNGQPENNYKTTPPVLDSDGSFFLYSRLTVDKSRWQEGNVFSCSVMHEALHNHYTQKSLSLSLG

SEQ ID NO: 121 - protein, 448 aa, artificial sequence
  Synthetic
QVQLQESGPGLVKPSETLSLTCAVSGYSISSGYYWGWIRQPPGKGLEWIGSIYHSGSTYYNPSLKSRVTISVDTSKNQFSLKLSSVTAADTAVYYCARASIYTPPPEYFQHWGQGTLVTVSSASTKGPSVFPLAPCSRSTSESTAALGCLVKDYFPEPVTVSWNSGALTSGVHTFPAVLQSSGLYSLSSVVTVPSSSLGTKTYTCNVDHKPSNTKVDKRVESKYGPPCPPCPAPEAAGGPSVFLFPPKPKDTLMISRTPEVTCVVVDVSQEDPEVQFNWYVDGVEVHNAKTKPREEQFNSTYRVVSVLTVLHQDWLNGKEYKCKVSNKGLPSSIEKTISKAKGQPREPQVYTLPPSQEEMTKNQVSLTCLVKGFYPSDIAVEWESNGQPENNYKTTPPVLDSDGSFFLYSRLTVDKSRWQEGNVFSCSVMHEALHNHYTQKSLSLSLG

SEQ ID NO: 122 - protein, 448 aa, artificial sequence
  Synthetic
QVQLQESGPGLVKPSETLSLTCAVSGYSISEGYYWGWIRQPPGKGLEWIGSIYHTGFTYYNPSLKSRVTISVDTSKNQFSLKLSSVTAADTAVYYCARASIYTPPPEYFQHWGQGTLVTVSSASTKGPSVFPLAPCSRSTSESTAALGCLVKDYFPEPVTVSWNSGALTSGVHTFPAVLQSSGLYSLSSVVTVPSSSLGTKTYTCNVDHKPSNTKVDKRVESKYGPPCPPCPAPEAAGGPSVFLFPPKPKDTLMISRTPEVTCVVVDVSQEDPEVQFNWYVDGVEVHNAKTKPREEQFNSTYRVVSVLTVLHQDWLNGKEYKCKVSNKGLPSSIEKTISKAKGQPREPQVYTLPPSQEEMTKNQVSLTCLVKGFYPSDIAVEWESNGQPENNYKTTPPVLDSDGSFFLYSRLTVDKSRWQEGNVFSCSVMHEALHNHYTQKSLSLSLG

SEQ ID NO: 123 - protein, 448 aa, artificial sequence
  Synthetic
QVQLQESGPGLVKPSETLSLTCAVSGYSISSGYYWAWIRQPPGKGLEWIGSIFHSGFTFYNPSLKSRVTISVDTSKNQFSLKLSSVTAADTAVYYCARASIYTPPPEYFQHWGQGTLVTVSSASTKGPSVFPLAPCSRSTSESTAALGCLVKDYFPEPVTVSWNSGALTSGVHTFPAVLQSSGLYSLSSVVTVPSSSLGTKTYTCNVDHKPSNTKVDKRVESKYGPPCPPCPAPEAAGGPSVFLFPPKPKDTLMISRTPEVTCVVVDVSQEDPEVQFNWYVDGVEVHNAKTKPREEQFNSTYRVVSVLTVLHQDWLNGKEYKCKVSNKGLPSSIEKTISKAKGQPREPQVYTLPPSQEEMTKNQVSLTCLVKGFYPSDIAVEWESNGQPENNYKTTPPVLDSDGSFFLYSRLTVDKSRWQEGNVFSCSVMHEALHNHYTQKSLSLSLG

SEQ ID NO: 124 - protein, 214 aa, artificial sequence
  Synthetic
DIQMTQSPSSLSASVGDRVTITCQASQDITNYLNWYQQKPGKAPKLLIYDASNLETGVPSRFSGSGSGTDFTFTISSLQPEDIATYYCQQSVVLPFTFGGGTKVEIKRTVAAPSVFIFPPSDEQLKSGTASVVCLLNNFYPREAKVQWKVDNALQSGNSQESVTEQDSKDSTYSLSSTLTLSKADYEKHKVYACEVTHQGLSSPVTKSFNRGEC

SEQ ID NO: 125 - protein, 216 aa, artificial sequence
  Synthetic
EIVLTQSPGTLSLSPGERATLSCRASQSVSSSYLAWYQQKPGQAPRLLIYGASSRATGIPDRFSGSGSGTDFTLTISRLEPEDFAVYYCQQYYDYPPITFGGGTKVEIKRTVAAPSVFIFPPSDEQLKSGTASVVCLLNNFYPREAKVQWKVDNALQSGNSQESVTEQDSKDSTYSLSSTLTLSKADYEKHKVYACEVTHQGLSSPVTKSFNRGEC

SEQ ID NO: 126 - protein, 213 aa, artificial sequence
  Synthetic
EIVMTQSPATLSVSPGERATLSCRASQSVSSNLAWYQQKPGQAPRLLIYGASTRATGIPARFSGSGSGTEFTLTISSLQSEDFAVYYCQQYTNHYTFGGGTKVEIKRTVAAPSVFIFPPSDEQLKSGTASVVCLLNNFYPREAKVQWKVDNALQSGNSQESVTEQDSKDSTYSLSSTLTLSKADYEKHKVYACEVTHQGLSSPVTKSFNRGEC

SEQ ID NO: 127 - protein, 214 aa, artificial sequence
  Synthetic
DIQLTQSPSSVSASVGDRVTITCRASQDISSWLAWYQQKPGKAPKLLIYAASSLQSGVPSRFSGSGSGTDFTLTISSLQPEDFATYYCQQANDFPITFGGGTKVEIKRTVAAPSVFIFPPSDEQLKSGTASVVCLLNNFYPREAKVQWKVDNALQSGNSQESVTEQDSKDSTYSLSSTLTLSKADYEKHKVYACEVTHQGLSSPVTKSFNRGEC

SEQ ID NO: 128 - protein, 215 aa, artificial sequence
  Synthetic
EIVLTQSPGTLSLSPGERATLSCRASQSVSSSYLAWYQQKPGQAPRLLIYGASSRATGIPDRFSGSGSGTDFTLTISRLEPEDFAVYYCQQYVLYPFTFGGGTKVEIKRTVAAPSVFIFPPSDEQLKSGTASVVCLLNNFYPREAKVQWKVDNALQSGNSQESVTEQDSKDSTYSLSSTLTLSKADYEKHKVYACEVTHQGLSSPVTKSFNRGEC

SEQ ID NO: 129 - protein, 215 aa, artificial sequence
  Synthetic
EIVLTQSPGTLSLSPGERATLSCGASQSVSSSYLAWYQQKPGQAPRLLIYGASSRATGIPDRFSGSGSGTDFTLTISRLEPEDFAVYYCQQYVLYPFTFGGGTKVEIKRTVAAPSVFIFPPSDEQLKSGTASVVCLLNNFYPREAKVQWKVDNALQSGNSQESVTEQDSKDSTYSLSSTLTLSKADYEKHKVYACEVTHQGLSSPVTKSFNRGEC

SEQ ID NO: 130 - protein, 213 aa, artificial sequence
  Synthetic
DIQMTQSPSTLSASVGDRVTITCRASQSISSWLAWYQQKPGKAPKLLIYDASSLESGVPSRFSGSGSGTEFTLTISSLQPDDFATYYCQQSRIYSTFGGGTKVEIKRTVAAPSVFIFPPSDEQLKSGTASVVCLLNNFYPREAKVQWKVDNALQSGNSQESVTEQDSKDSTYSLSSTLTLSKADYEKHKVYACEVTHQGLSSPVTKSFNRGEC

SEQ ID NO: 131 - protein, 574 aa, artificial sequence
  Synthetic
MCPRAARAPATLLLALGAVLWPAAGAWELTILHTNDVHSRLEQTSEDSSKCVNASRCMGGVARLFTKVQQIRRAEPNVLLLDAGDQYQGTIWFTVYKGAEVAHFMNALRYDAMALGNHEFDNGVEGLIEPLLKEAKFPILSANIKAKGPLASQISGLYLPYKVLPVGDEVVGIVGYTSKETPFLSNPGTNLVFEDEITALQPEVDKLKTLNVNKIIALGHSGFEMDKLIAQKVRGVDVVVGGHSNTFLYTGNPPSKEVPAGKYPFIVTSDDGRKVPVVQAYAFGKYLGYLKIEFDERGNVISSHGNPILLNSSIPEDPSIKADINKWRIKLDNYSTQELGKTIVYLDGSSQSCRFRECNMGNLICDAMINNNLRHTDEMFWNHVSMCILNGGGIRSPIDERNNGTITWENLAAVLPFGGTFDLVQLKGSTLKKAFEHSVHRYGQSTGEFLQVGGIHVVYDLSRKPGDRVVKLDVLCTKCRVPSYDPLKMDEVYKVILPNFLANGGDGFQMIKDELLRHDSGDQDINVVSTYISKMKVIYPAVEGRIKFSTGSHCHGSFSLIFLSLWAVIFVLYQ

SEQ ID NO: 132 - protein, 10 aa, artificial sequence
  Synthetic
  misc_feature (5)..(5): Xaa can be Asp、Ser、His、Leu、Asn
  misc_feature (6)..(6): Xaa can be Asp、Asn、Ser、Phe、His
  misc_feature (7)..(7): Xaa can be Tyr、Phe、Leu
  misc_feature (8)..(8): Xaa can be Ala、Tyr、Phe、Gly、Ser
  misc_feature (10)..(10): Xaa can be His、Ser、Thr、Ala
GFTFXXXXMX

SEQ ID NO: 133 - protein, 11 aa, artificial sequence
  Synthetic
  misc_feature (6)..(6): Xaa can be Ser、Glu
  misc_feature (11)..(11): Xaa can be Gly 、Ala
GYSISXGYYWX

SEQ ID NO: 134 - protein, 17 aa, artificial sequence
  Synthetic
  misc_feature (1)..(1): Xaa can be Gly、Ala、Val、His
  misc_feature (3)..(3): Xaa can be Ser、Asn、deletion
  misc_feature (4)..(4): Xaa can be Trp 、Gly、Tyr、Asp、Val
  misc_feature (5)..(5): Xaa can be Ser、Arg 、Thr、Glu
  misc_feature (6)..(6): Xaa can be Ser、Gly、Ala
  misc_feature (7)..(7): Xaa can be Gly、Thr、Ser、Arg 、Ile
  misc_feature (8)..(8): Xaa can be Ser、Pro、Ala、Asn、Asp
  misc_feature (9)..(9): Xaa can be Ile、Thr、Lys
  misc_feature (10)..(10): Xaa can be Gly、Asp、Tyr
XIXXXXXXXXYADSVKG

SEQ ID NO: 135 - protein, 16 aa, artificial sequence
  Synthetic
  misc_feature (3)..(3): Xaa can be Tyr、Phe
  misc_feature (5)..(5): Xaa can be Ser、Thr
  misc_feature (7)..(7): Xaa can be Ser、Phe
  misc_feature (9)..(9): Xaa can be Tyr、Phe
SIXHXGXTXYNPSLKS

SEQ ID NO: 136 - protein, 5 aa, artificial sequence
  Synthetic
DYAMH

SEQ ID NO: 137 - protein, 5 aa, artificial sequence
  Synthetic
DFYMH

SEQ ID NO: 138 - protein, 5 aa, artificial sequence
  Synthetic
DYFMH

SEQ ID NO: 139 - protein, 5 aa, artificial sequence
  Synthetic
NYAMS

SEQ ID NO: 140 - protein, 5 aa, artificial sequence
  Synthetic
NYAMT

SEQ ID NO: 141 - protein, 5 aa, artificial sequence
  Synthetic
NLAMS

SEQ ID NO: 142 - protein, 5 aa, artificial sequence
  Synthetic
NYAMA

SEQ ID NO: 143 - protein, 5 aa, artificial sequence
  Synthetic
SYGMH

SEQ ID NO: 144 - protein, 5 aa, artificial sequence
  Synthetic
FYGMH

SEQ ID NO: 145 - protein, 5 aa, artificial sequence
  Synthetic
HYGMH

SEQ ID NO: 146 - protein, 5 aa, artificial sequence
  Synthetic
SYSMH

SEQ ID NO: 147 - protein, 6 aa, artificial sequence
  Synthetic
SGYYWG

SEQ ID NO: 148 - protein, 6 aa, artificial sequence
  Synthetic
EGYYWG

SEQ ID NO: 149 - protein, 6 aa, artificial sequence
  Synthetic
SGYYWA

SEQ ID NO: 150 - protein, 12 aa, artificial sequence
  Synthetic
DRRYGLTYGMDV

SEQ ID NO: 151 - protein, 11 aa, artificial sequence
  Synthetic
GKYLPTGSVDY

SEQ ID NO: 152 - protein, 15 aa, artificial sequence
  Synthetic
GGPYGSGSYWDTFDY

SEQ ID NO: 153 - protein, 11 aa, artificial sequence
  Synthetic
GGARYPIAFDI

SEQ ID NO: 154 - protein, 11 aa, artificial sequence
  Synthetic
GWLRYPIAFDI

SEQ ID NO: 155 - protein, 10 aa, artificial sequence
  Synthetic
SRYDWSLFDI

SEQ ID NO: 156 - protein, 13 aa, artificial sequence
  Synthetic
ASIYTPPPEYFQH